European Patent Application EP 4 115 911 A1, published January 11, 2023. Title: STABILIZED FIBRONECTIN DOMAIN COMPOSITIONS, METHODS AND USES. Applicant: JANSSEN BIOTECH, INC. The sequence listing filed with the application follows.

SEQUENCE LISTING (151 sequences)

SEQ ID NO: 1 - protein, 87 aa, Homo sapiens
SPPKDLVVTEVTEETVNLAWDNEMRVTEYLVVYTPTHEGGLEMQFRVPGDQTSTIIQELEPGVEYFIRVFAILENKKSIPVSARVAT

SEQ ID NO: 2 - protein, 95 aa, Homo sapiens
TYLPAPEGLKFKSIKETSVEVEWDPLDIAFETWEIIFRNMNKEDEGEITKSLRRPETSYRQTGLAPGQEYEISLHIVKNNTRGPGLKRVTTTRLD

SEQ ID NO: 3 - protein, 88 aa, Homo sapiens
DAPSQIEVKDVTDTTALITWFKPLAEIDGIELTYGIKDVPGDRTTIDLTEDENQYSIGNLKPDTEYEVSLISRRGDMSSNPAKETFTT

SEQ ID NO: 4 - protein, 100 aa, Homo sapiens
TGLDAPRNLRRVSQTDNSITLEWRNGKAAIDSYRIKYAPISGGDHAEVDVPKSQQATTKTTLTGLRPGTEYGIGVSAVKEDKESNPATINAATELDTPKD

SEQ ID NO: 5 - protein, 88 aa, Homo sapiens
DTPKDLQVSETAETSLTLLWKTPLAKFDRYRLNYSLPTGQWVGVQLPRNTTSYVLRGLEPGQEYNVLLTAEKGRHKSKPAKSKPARVK

SEQ ID NO: 6 - protein, 92 aa, Homo sapiens
QAPELENLTVTEVGWDGLRLNWTAADQAYEHFIIQVQEANKVEAARNLTVPGSLRAVDIPGLKAATPYTVSIYGVIQGYRTPVLSAEASTGE

SEQ ID NO: 7 - protein, 91 aa, Homo sapiens
ETPNLGEVVVAEVGWDALKLNWTAPEGAYEYFFIQVQEADTVEAAQNLTVPGGLRSTDLPGLKAATHYTITIRGVTQDFSTTPLSVEVLTE

SEQ ID NO: 8 - protein, 91 aa, Homo sapiens
EVPDMGNLTVTEVSWDALRLNWTTPDGTYDQFTIQVQEADQVEEAHNLTVPGSLRSMEIPGLRAGTPYTVTLHGEVRGHSTRPLAVEVVTE

SEQ ID NO: 9 - protein, 95 aa, Homo sapiens
DLPQLGDLAVSEVGWDGLRLNWTAADNAYEHFVIQVQEVNKVEAAQNLTLPGSLRAVDIPGLEAATPYRVSIYGVIRGYRTPVLSAEASTAKEPE

SEQ ID NO: 10 - protein, 91 aa, Homo sapiens
KEPEIGNLNVSDITPESFNLSWMATDGIFETFTIEIIDSNRLLETVEYNISGAERTAHISGLPPSTDFIVYLSGLAPSIRTKTISATATTE

SEQ ID NO: 11 - protein, 91 aa, Homo sapiens
ALPLLENLTISDINPYGFTVSWMASENAFDSFLVTVVDSGKLLDPQEFTLSGTQRKLELRGLITGIGYEVMVSGFTQGHQTKPLRAEIVTE

SEQ ID NO: 12 - protein, 92 aa, Homo sapiens
AEPEVDNLLVSDATPDGFRLSWTADEGVFDNFVLKIRDTKKQSEPLEITLLAPERTRDLTGLREATEYEIELYGISKGRRSQTVSAIATTAM

SEQ ID NO: 13 - protein, 89 aa, Homo sapiens
GSPKEVIFSDITENSATVSWRAPTAQVESFRITYVPITGGTPSMVTVDGTKTQTRLVKLIPGVEYLVSIIAMKGFEESEPVSGSFTTAL

SEQ ID NO: 14 - protein, 88 aa, Homo sapiens
DGPSGLVTANITDSEALARWQPAIATVDSYVISYTGEKVPEITRTVSGNTVEYALTDLEPATEYTLRIFAEKGPQKSSTITAKFTTDL

SEQ ID NO: 15 - protein, 89 aa, Homo sapiens
DSPRDLTATEVQSETALLTWRPPRASVTGYLLVYESVDGTVKEVIVGPDTTSYSLADLSPSTHYTAKIQALNGPLRSNMIQTIFTTIGL

SEQ ID NO: 16 - protein, 89 aa, Artificial Sequence
  Binding polypeptide
LPAPKNLVVSEVTEDSLRLSWTAPDAAFDSFLIQYQESEKVGEAINLTVPGSERSYDLTGLKPGTEYTVSIYGVKGGHRSNPLSAEFTT

SEQ ID NO: 17 - DNA, 267 bp, Artificial Sequence
  Nucleotide encoding binding polynucleotide
ctgccggcgccgaaaaacctggttgtttctgaagttaccgaagactctctgcgtctgtcttggaccgcgccggacgcggcgttcgactctttcctgatccagtaccaggaatctgaaaaagttggtgaagcgatcaacctgaccgttccgggttctgaacgttcttacgacctgaccggtctgaaaccgggtaccgaatacaccgtttctatctacggtgttaaaggtggtcaccgttctaacccgctgtctgcggaattcaccacc

SEQ ID NO: 18 - DNA, 68 bp, Artificial Sequence
  unknown (28)(29)(31)(32)(34)(35)(37)(38)(40)(41)(43)(44)(46)(47): Primer wherein n can be represented by a, c, t or g
gaatacaccgtttctatctacggtgttnnsnnsnnsnnsnnsnnsnnsccgctgtctgcggaattcac

SEQ ID NO: 19 - DNA, 64 bp, Artificial Sequence
  unknown (22)(23)(25)(26)(28)(29)(31)(32)(34)(35)(37)(38): Primer wherein n can be represented by a, c, t or g
gactctctgcgtctgtcttggnnsnnsnnsnnsnnsnnsttcgactctttcctgatccagtacc

SEQ ID NO: 20 - DNA, 63 bp, Artificial Sequence
  unknown (21)(22)(23)(24)(25)(26)(27)(28)(29)(30)(31)(32)(33)(34)(35)(36)(37)(38)(39)(40)(41): Primer wherein n can be represented by a, c, t or g and s can be represented by g or c.
gtgaattccgcagacagcggsnnsnnsnnsnnsnnsnnsnnaacaccgtagatagaaacggtg

SEQ ID NO: 21 - protein, 6 aa, Artificial Sequence
  Protein Scaffold Based On A Human Fibronectin Type III (FN3) Domain Sequence
SYGFNN

SEQ ID NO: 22 - protein, 6 aa, Artificial Sequence
  Protein Scaffold Based On A Human Fibronectin Type III (FN3) Domain Sequence
TYEGES

SEQ ID NO: 23 - protein, 6 aa, Artificial Sequence
  Protein Scaffold Based On A Human Fibronectin Type III (FN3) Domain Sequence
TYESES

SEQ ID NO: 24 - protein, 6 aa, Artificial Sequence
  Protein Scaffold Based On A Human Fibronectin Type III (FN3) Domain Sequence
TNWMDS

SEQ ID NO: 25 - protein, 6 aa, Artificial Sequence
  Protein Scaffold Based On A Human Fibronectin Type III (FN3) Domain Sequence
KSVFIM

SEQ ID NO: 26 - protein, 6 aa, Artificial Sequence
  Protein Scaffold Based On A Human Fibronectin Type III (FN3) Domain Sequence
YSSYAT

SEQ ID NO: 27 - protein, 6 aa, Artificial Sequence
  Protein Scaffold Based On A Human Fibronectin Type III (FN3) Domain Sequence
RFHPFP

SEQ ID NO: 28 - protein, 6 aa, Artificial Sequence
  Protein Scaffold Based On A Human Fibronectin Type III (FN3) Domain Sequence
MMCMPL

SEQ ID NO: 29 - protein, 6 aa, Artificial Sequence
  Protein Scaffold Based On A Human Fibronectin Type III (FN3) Domain Sequence
YCRVRD

SEQ ID NO: 30 - protein, 6 aa, Artificial Sequence
  Protein Scaffold Based On A Human Fibronectin Type III (FN3) Domain Sequence
MDCFMG

SEQ ID NO: 31 - protein, 6 aa, Artificial Sequence
  Protein Scaffold Based On A Human Fibronectin Type III (FN3) Domain Sequence
TYRFNS

SEQ ID NO: 32 - protein, 6 aa, Artificial Sequence
  Protein Scaffold Based On A Human Fibronectin Type III (FN3) Domain Sequence
ASRRSL

SEQ ID NO: 33 - protein, 6 aa, Artificial Sequence
  Protein Scaffold Based On A Human Fibronectin Type III (FN3) Domain  Sequence
TIESES

SEQ ID NO: 34 - protein, 5 aa, Artificial Sequence
  Protein Scaffold Based On A Human Fibronectin Type III (FN3) Domain Sequence
TLMQS

SEQ ID NO: 35 - protein, 6 aa, Artificial Sequence
  Protein Scaffold Based On A Human Fibronectin Type III (FN3) Domain Sequence
IYDSES

SEQ ID NO: 36 - protein, 6 aa, Artificial Sequence
  Protein Scaffold Based On A Human Fibronectin Type III (FN3) Domain Sequence
DRKRFI

SEQ ID NO: 37 - protein, 6 aa, Artificial Sequence
  Protein Scaffold Based On A Human Fibronectin Type III (FN3) Domain Sequence
EFWRGS

SEQ ID NO: 38 - protein, 6 aa, Artificial Sequence
  Protein Scaffold Based On A Human Fibronectin Type III (FN3) Domain Sequence
GLLDPL

SEQ ID NO: 39 - protein, 6 aa, Artificial Sequence
  Protein Scaffold Based On A Human Fibronectin Type III (FN3) Domain Sequence
GLVLPE

SEQ ID NO: 40 - protein, 6 aa, Artificial Sequence
  Protein Scaffold Based On A Human Fibronectin Type III (FN3) Domain Sequence
MASDGL

SEQ ID NO: 41 - protein, 6 aa, Artificial Sequence
  Protein Scaffold Based On A Human Fibronectin Type III (FN3) Domain Sequence
NKTETN

SEQ ID NO: 42 - protein, 6 aa, Artificial Sequence
  Protein Scaffold Based On A Human Fibronectin Type III (FN3) Domain Sequence
QAERKV

SEQ ID NO: 43 - protein, 6 aa, Artificial Sequence
  Protein Scaffold Based On A Human Fibronectin Type III (FN3) Domain Sequence
SQVCTL

SEQ ID NO: 44 - protein, 6 aa, Artificial Sequence
  Protein Scaffold Based On A Human Fibronectin Type III (FN3) Domain Sequence
YFDKDS

SEQ ID NO: 45 - protein, 6 aa, Artificial Sequence
  Protein Scaffold Based On A Human Fibronectin Type III (FN3) Domain Sequence
YFECEP

SEQ ID NO: 46 - protein, 7 aa, Artificial Sequence
  Protein Scaffold Based On A Human Fibronectin Type III (FN3) Domain Sequence
QIGPIIP

SEQ ID NO: 47 - protein, 7 aa, Artificial Sequence
  Protein Scaffold Based On A Human Fibronectin Type III (FN3) Domain Sequence
SIRTIDS

SEQ ID NO: 48 - protein, 7 aa, Artificial Sequence
  Protein Scaffold Based On A Human Fibronectin Type III (FN3) Domain Sequence
PKFHSPL

SEQ ID NO: 49 - protein, 7 aa, Artificial Sequence
  Protein Scaffold Based On A Human Fibronectin Type III (FN3) Domain Sequence
WKTTIWF

SEQ ID NO: 50 - protein, 7 aa, Artificial Sequence
  Protein Scaffold Based On A Human Fibronectin Type III (FN3) Domain Sequence
RKNWKTR

SEQ ID NO: 51 - protein, 7 aa, Artificial Sequence
  Protein Scaffold Based On A Human Fibronectin Type III (FN3) Domain Sequence
RLFRIYQ

SEQ ID NO: 52 - protein, 7 aa, Artificial Sequence
  Protein Scaffold Based On A Human Fibronectin Type III (FN3) Domain Sequence
WLSRSYD

SEQ ID NO: 53 - protein, 7 aa, Artificial Sequence
  Protein Scaffold Based On A Human Fibronectin Type III (FN3) Domain Sequence
WLSRSCD

SEQ ID NO: 54 - protein, 7 aa, Artificial Sequence
  Protein Scaffold Based On A Human Fibronectin Type III (FN3) Domain Sequence
WMGPYCD

SEQ ID NO: 55 - protein, 7 aa, Artificial Sequence
  Protein Scaffold Based On A Human Fibronectin Type III (FN3) Domain Sequence
RRRRYSF

SEQ ID NO: 56 - protein, 7 aa, Artificial Sequence
  Protein Scaffold Based On A Human Fibronectin Type III (FN3) Domain Sequence
HIVPMVP

SEQ ID NO: 57 - protein, 7 aa, Artificial Sequence
  Protein Scaffold Based On A Human Fibronectin Type III (FN3) Domain Sequence
QIEPIIR

SEQ ID NO: 58 - protein, 7 aa, Artificial Sequence
  Protein Scaffold Based On A Human Fibronectin Type III (FN3) Domain Sequence
PSAANNP

SEQ ID NO: 59 - protein, 7 aa, Artificial Sequence
  Protein Scaffold Based On A Human Fibronectin Type III (FN3) Domain Sequence
VRLRYVQ

SEQ ID NO: 60 - protein, 7 aa, Artificial Sequence
  Protein Scaffold Based On A Human Fibronectin Type III (FN3) Domain Sequence
QVGPLIP

SEQ ID NO: 61 - protein, 7 aa, Artificial Sequence
  Protein Scaffold Based On A Human Fibronectin Type III (FN3) Domain Sequence
RIGPILP

SEQ ID NO: 62 - protein, 7 aa, Artificial Sequence
  Protein Scaffold Based On A Human Fibronectin Type III (FN3) Domain Sequence
QIGPLLP

SEQ ID NO: 63 - protein, 7 aa, Artificial Sequence
  Protein Scaffold Based On A Human Fibronectin Type III (FN3) Domain Sequence
RIGPLLP

SEQ ID NO: 64 - protein, 7 aa, Artificial Sequence
  Protein Scaffold Based On A Human Fibronectin Type III (FN3) Domain Sequence
QVGPLLP

SEQ ID NO: 65 - protein, 7 aa, Artificial Sequence
  Protein Scaffold Based On A Human Fibronectin Type III (FN3) Domain Sequence
RIGPMLP

SEQ ID NO: 66 - protein, 7 aa, Artificial Sequence
  Protein Scaffold Based On A Human Fibronectin Type III (FN3) Domain Sequence
QIGPVLP

SEQ ID NO: 67 - protein, 7 aa, Artificial Sequence
  Protein Scaffold Based On A Human Fibronectin Type III (FN3) Domain Sequence
RIGPVLP

SEQ ID NO: 68 - protein, 7 aa, Artificial Sequence
  Protein Scaffold Based On A Human Fibronectin Type III (FN3) Domain Sequence
QIGPMMP

SEQ ID NO: 69 - protein, 7 aa, Artificial Sequence
  Protein Scaffold Based On A Human Fibronectin Type III (FN3) Domain Sequence
QVGPLVP

SEQ ID NO: 70 - protein, 7 aa, Artificial Sequence
  Protein Scaffold Based On A Human Fibronectin Type III (FN3) Domain Sequence
QIGPMLP

SEQ ID NO: 71 - protein, 7 aa, Artificial Sequence
  Protein Scaffold Based On A Human Fibronectin Type III (FN3) Domain Sequence
QVGPILP

SEQ ID NO: 72 - protein, 7 aa, Artificial Sequence
  Protein Scaffold Based On A Human Fibronectin Type III (FN3) Domain Sequence
QVGPMLP

SEQ ID NO: 73 - protein, 7 aa, Artificial Sequence
  Protein Scaffold Based On A Human Fibronectin Type III (FN3) Domain Sequence
QIGPIVP

SEQ ID NO: 74 - protein, 7 aa, Artificial Sequence
  Protein Scaffold Based On A Human Fibronectin Type III (FN3) Domain Sequence
MIGPLLP

SEQ ID NO: 75 - protein, 7 aa, Artificial Sequence
  Protein Scaffold Based On A Human Fibronectin Type III (FN3) Domain Sequence
QIGPLFP

SEQ ID NO: 76 - protein, 7 aa, Artificial Sequence
  Protein Scaffold Based On A Human Fibronectin Type III (FN3) Domain Sequence
QIGPMVP

SEQ ID NO: 77 - protein, 7 aa, Artificial Sequence
  Protein Scaffold Based On A Human Fibronectin Type III (FN3) Domain Sequence
QIGPIVP

SEQ ID NO: 78 - protein, 7 aa, Artificial Sequence
  Protein Scaffold Based On A Human Fibronectin Type III (FN3) Domain Sequence
RIEPILP

SEQ ID NO: 79 - protein, 7 aa, Artificial Sequence
  Protein Scaffold Based On A Human Fibronectin Type III (FN3) Domain Sequence
VAGSVWP

SEQ ID NO: 80 - protein, 7 aa, Artificial Sequence
  Protein Scaffold Based On A Human Fibronectin Type III (FN3) Domain Sequence
REGATLY

SEQ ID NO: 81 - protein, 7 aa, Artificial Sequence
  Protein Scaffold Based On A Human Fibronectin Type III (FN3) Domain Sequence
KQIPPIL

SEQ ID NO: 82 - protein, 7 aa, Artificial Sequence
  Protein Scaffold Based On A Human Fibronectin Type III (FN3) Domain Sequence
LSLSSVL

SEQ ID NO: 83 - protein, 7 aa, Artificial Sequence
  Protein Scaffold Based On A Human Fibronectin Type III (FN3) Domain Sequence
HMLLPLP

SEQ ID NO: 84 - protein, 7 aa, Artificial Sequence
  Protein Scaffold Based On A Human Fibronectin Type III (FN3) Domain Sequence
MIGPLIP

SEQ ID NO: 85 - protein, 7 aa, Artificial Sequence
  Protein Scaffold Based On A Human Fibronectin Type III (FN3) Domain Sequence
TIGPHIP

SEQ ID NO: 86 - protein, 7 aa, Artificial Sequence
  Protein Scaffold Based On A Human Fibronectin Type III (FN3) Domain Sequence
EIGPCLP

SEQ ID NO: 87 - protein, 7 aa, Artificial Sequence
  Protein Scaffold Based On A Human Fibronectin Type III (FN3) Domain Sequence
EIGPVLP

SEQ ID NO: 88 - protein, 7 aa, Artificial Sequence
  Protein Scaffold Based On A Human Fibronectin Type III (FN3) Domain Sequence
KIGPCLP

SEQ ID NO: 89 - protein, 7 aa, Artificial Sequence
  Protein Scaffold Based On A Human Fibronectin Type III (FN3) Domain Sequence
MIGPVLP

SEQ ID NO: 90 - protein, 7 aa, Artificial Sequence
  Protein Scaffold Based On A Human Fibronectin Type III (FN3) Domain Sequence
QIGPILP

SEQ ID NO: 91 - protein, 7 aa, Artificial Sequence
  Protein Scaffold Based On A Human Fibronectin Type III (FN3) Domain Sequence
EVGPILP

SEQ ID NO: 92 - protein, 7 aa, Artificial Sequence
  Protein Scaffold Based On A Human Fibronectin Type III (FN3) Domain Sequence
QVGPLLP

SEQ ID NO: 93 - protein, 7 aa, Artificial Sequence
  Protein Scaffold Based On A Human Fibronectin Type III (FN3) Domain Sequence
QIGPVMP

SEQ ID NO: 94 - protein, 7 aa, Artificial Sequence
  Protein Scaffold Based On A Human Fibronectin Type III (FN3) Domain Sequence
QIGPCVP

SEQ ID NO: 95 - protein, 7 aa, Artificial Sequence
  Protein Scaffold Based On A Human Fibronectin Type III (FN3) Domain Sequence
QIGPLVP

SEQ ID NO: 96 - protein, 7 aa, Artificial Sequence
  Protein Scaffold Based On A Human Fibronectin Type III (FN3) Domain Sequence
RGLVMPM

SEQ ID NO: 97 - protein, 7 aa, Artificial Sequence
  Protein Scaffold Based On A Human Fibronectin Type III (FN3) Domain Sequence
MIGPILP

SEQ ID NO: 98 - protein, 7 aa, Artificial Sequence
  Protein Scaffold Based On A Human Fibronectin Type III (FN3) Domain Sequence
CIGPMVP

SEQ ID NO: 99 - protein, 7 aa, Artificial Sequence
  Protein Scaffold Based On A Human Fibronectin Type III (FN3) Domain Sequence
FIGPVLP

SEQ ID NO: 100 - protein, 7 aa, Artificial Sequence
  Protein Scaffold Based On A Human Fibronectin Type III (FN3) Domain Sequence
HIGPILP

SEQ ID NO: 101 - protein, 7 aa, Artificial Sequence
  Protein Scaffold Based On A Human Fibronectin Type III (FN3) Domain Sequence
HIGPIMP

SEQ ID NO: 102 - protein, 7 aa, Artificial Sequence
  Protein Scaffold Based On A Human Fibronectin Type III (FN3) Domain Sequence
HIGPYLP

SEQ ID NO: 103 - protein, 7 aa, Artificial Sequence
  Protein Scaffold Based On A Human Fibronectin Type III (FN3) Domain Sequence
HVGPILP

SEQ ID NO: 104 - protein, 7 aa, Artificial Sequence
  Protein Scaffold Based On A Human Fibronectin Type III (FN3) Domain Sequence
IIGPLLP

SEQ ID NO: 105 - protein, 7 aa, Artificial Sequence
  Protein Scaffold Based On A Human Fibronectin Type III (FN3) Domain Sequence
MVGPLLP

SEQ ID NO: 106 - protein, 7 aa, Artificial Sequence
  Protein Scaffold Based On A Human Fibronectin Type III (FN3) Domain Sequence
MVGPLLP

SEQ ID NO: 107 - protein, 7 aa, Artificial Sequence
  Protein Scaffold Based On A Human Fibronectin Type III (FN3) Domain Sequence
NIGPYLP

SEQ ID NO: 108 - protein, 7 aa, Artificial Sequence
  Protein Scaffold Based On A Human Fibronectin Type III (FN3) Domain Sequence
NIGPYLP

SEQ ID NO: 109 - protein, 7 aa, Artificial Sequence
  Protein Scaffold Based On A Human Fibronectin Type III (FN3) Domain  Sequence
QIGPHLP

SEQ ID NO: 110 - protein, 7 aa, Artificial Sequence
  Protein Scaffold Based On A Human Fibronectin Type III (FN3) Domain Sequence
QIGPILG

SEQ ID NO: 111 - protein, 7 aa, Artificial Sequence
  Protein Scaffold Based On A Human Fibronectin Type III (FN3) Domain Sequence
QIGPILS

SEQ ID NO: 112 - protein, 7 aa, Artificial Sequence
  Protein Scaffold Based On A Human Fibronectin Type III (FN3) Domain Sequence
QIGPILT

SEQ ID NO: 113 - protein, 7 aa, Artificial Sequence
  Protein Scaffold Based On A Human Fibronectin Type III (FN3) Domain  Sequence
QIGPIMP

SEQ ID NO: 114 - protein, 7 aa, Artificial Sequence
  Protein Scaffold Based On A Human Fibronectin Type III (FN3) Domain Sequence
QIGPIPI

SEQ ID NO: 115 - protein, 7 aa, Artificial Sequence
  Protein Scaffold Based On A Human Fibronectin Type III (FN3) Domain Sequence
QIGPLLN

SEQ ID NO: 116 - protein, 7 aa, Artificial Sequence
  Protein Scaffold Based On A Human Fibronectin Type III (FN3) Domain Sequence
QIGPVFP

SEQ ID NO: 117 - protein, 7 aa, Artificial Sequence
  Protein Scaffold Based On A Human Fibronectin Type III (FN3) Domain Sequence
QIGPVLS

SEQ ID NO: 118 - protein, 7 aa, Artificial Sequence
  Protein Scaffold Based On A Human Fibronectin Type III (FN3) Domain Sequence
QIGPWLP

SEQ ID NO: 119 - protein, 7 aa, Artificial Sequence
  Protein Scaffold Based On A Human Fibronectin Type III (FN3) Domain Sequence
QVGPIMN

SEQ ID NO: 120 - protein, 7 aa, Artificial Sequence
  Protein Scaffold Based On A Human Fibronectin Type III (FN3) Domain Sequence
QVGPIMP

SEQ ID NO: 121 - protein, 7 aa, Artificial Sequence
  Protein Scaffold Based On A Human Fibronectin Type III (FN3) Domain Sequence
QVGPIVP

SEQ ID NO: 122 - protein, 7 aa, Artificial Sequence
  Protein Scaffold Based On A Human Fibronectin Type III (FN3) Domain Sequence
QVGPLLS

SEQ ID NO: 123 - protein, 7 aa, Artificial Sequence
  Protein Scaffold Based On A Human Fibronectin Type III (FN3) Domain Sequence
QVGPVLP

SEQ ID NO: 124 - protein, 7 aa, Artificial Sequence
  Protein Scaffold Based On A Human Fibronectin Type III (FN3) Domain Sequence
QVGPVLP

SEQ ID NO: 125 - protein, 7 aa, Artificial Sequence
  Protein Scaffold Based On A Human Fibronectin Type III (FN3) Domain Sequence
RIGPIMP

SEQ ID NO: 126 - protein, 7 aa, Artificial Sequence
  Protein Scaffold Based On A Human Fibronectin Type III (FN3) Domain Sequence
RIGPIVP

SEQ ID NO: 127 - protein, 7 aa, Artificial Sequence
  Protein Scaffold Based On A Human Fibronectin Type III (FN3) Domain Sequence
RIGPMFP

SEQ ID NO: 128 - protein, 7 aa, Artificial Sequence
  Protein Scaffold Based On A Human Fibronectin Type III (FN3) Domain Sequence
RIGPMIP

SEQ ID NO: 129 - protein, 7 aa, Artificial Sequence
  Protein Scaffold Based On A Human Fibronectin Type III (FN3) Domain Sequence
RIGPMVP

SEQ ID NO: 130 - protein, 7 aa, Artificial Sequence
  Protein Scaffold Based On A Human Fibronectin Type III (FN3) Domain Sequence
RIGPVIP

SEQ ID NO: 131 - protein, 7 aa, Artificial Sequence
  Protein Scaffold Based On A Human Fibronectin Type III (FN3) Domain Sequence
RVGPILP

SEQ ID NO: 132 - protein, 7 aa, Artificial Sequence
  Protein Scaffold Based On A Human Fibronectin Type III (FN3) Domain Sequence
RVGPLLP

SEQ ID NO: 133 - protein, 7 aa, Artificial Sequence
  Protein Scaffold Based On A Human Fibronectin Type III (FN3) Domain Sequence
TVGPHIP

SEQ ID NO: 134 - protein, 7 aa, Artificial Sequence
  Protein Scaffold Based On A Human Fibronectin Type III (FN3) Domain Sequence
PSWRSNW

SEQ ID NO: 135 - protein, 7 aa, Artificial Sequence
  Protein Scaffold Based On A Human Fibronectin Type III (FN3) Domain Sequence
ALRATLE

SEQ ID NO: 136 - protein, 7 aa, Artificial Sequence
  Protein Scaffold Based On A Human Fibronectin Type III (FN3) Domain Sequence
KYGYLTP

SEQ ID NO: 137 - protein, 7 aa, Artificial Sequence
  Protein Scaffold Based On A Human Fibronectin Type III (FN3) Domain Sequence
RIGPMLP

SEQ ID NO: 138 - protein, 7 aa, Artificial Sequence
  Protein Scaffold Based On A Human Fibronectin Type III (FN3) Domain Sequence
NPFCSRF

SEQ ID NO: 139 - protein, 7 aa, Artificial Sequence
  Protein Scaffold Based On A Human Fibronectin Type III (FN3) Domain Sequence
YYLHQWC

SEQ ID NO: 140 - protein, 7 aa, Artificial Sequence
  Protein Scaffold Based On A Human Fibronectin Type III (FN3) Domain Sequence
HIVPLLR

SEQ ID NO: 141 - protein, 7 aa, Artificial Sequence
  Protein Scaffold Based On A Human Fibronectin Type III (FN3) Domain Sequence
TSGGGGS

SEQ ID NO: 142 - protein, 89 aa, Artificial Sequence
  Binding polypeptide
LPAPKNLVVSEVTEDSLRLSWTAPDAAFDSFLIQYQESEKVGEAIVLTVPGSERSYDLTGLKPGTEYTVSIYGVKGGHRSNPLSAEFTT

SEQ ID NO: 143 - protein, 89 aa, Binding polypeptide
LPAPKNLVVSEVTPDSLRLSWTAPDAAFDSFLIQYQESEKVGEAINLTVPGSERSYDLTGLKPGTEYTVSIYGVKGGHRSNPLSAEFTT

SEQ ID NO: 144 - protein, 89 aa, Artificial Sequence
  Binding polypeptide
LPAPKNLVVSNVTEDSLRLSWTAPDAAFDSFLIQYQESEKVGEAINLTVPGSERSYDLTGLKPGTEYTVSIYGVKGGHRSNPLSAEFTT

SEQ ID NO: 145 - protein, 89 aa, Binding polypeptide
LPAPKNLVVSEVTEDSLRLSWTAPDAAFDSFLIQYQPSEKVGEAINLTVPGSERSYDLTGLKPGTEYTVSIYGVKGGHRSNPLSAEFTT

SEQ ID NO: 146 - protein, 89 aa, Artificial Sequence
  Binding polypeptide
LPAPKNLVVSEVTEDSLRLSWTAPDAAFDSFLIQYQESEKVGEAINLTVPGSERSYDLTGLKPGTEYTVSIYYVKGGHRSNPLSAEFTT

SEQ ID NO: 147 - protein, 89 aa, Artificial Sequence
  Binding polypeptide
LPAPKNLVVSEVTEDSLRLSWTAPDAAFDSFLIQYQESEKVGEAINLTVPGSERSYDLTGLKPGTEYTVSIYGVKGGHRSNPLSAIFTT

SEQ ID NO: 148 - protein, 89 aa, Artificial Sequence
  Binding polypeptide
LPAPKNLVVSEVTEDSLRLSWTAPDAAFDSFLIQYQESEKVGEAIVLTVPGSERSYDLTGLKPGTEYTVSIYGVKGGHRSNPLSAIFTT

SEQ ID NO: 149 - protein, 89 aa, Artificial Sequence
  Binding polypeptide
LPAPKNLVVSEVTPDSLRLSWTAPDAAFDSFLIQYQESEKVGEAIVLTVPGSERSYDLTGLKPGTEYTVSIYGVKGGHRSNPLSAIFTT

SEQ ID NO: 150 - protein, 89 aa, Artificial Sequence
  Binding polypeptide
LPAPKNLVVSEVTEDSARLSWTAPDAAFDSFLIQYQESEKVGEAIVLTVPGSERSYDLTGLKPGTEYTVSIYGVKGGHRSNPLSAIFTT

SEQ ID NO: 151 - protein, 89 aa, Artificial Sequence
  Binding polypeptide
LPAPKNLVVSEVTEDSARLSWTAPDAAFDSFLIQYQESEKVGEAINLTVPGSERSYDLTGLKPGTEYTVSIYGVKGGHRSNPLSAEFTT